European Patent Application EP 4 617 284 A1, published September 17, 2025. Title: ANTI-IL-13 LONG-ACTING NANOBODY SEQUENCE AND USE THEREOF. Applicant: SHANGHAI NOVAMAB BIOPHARMACEUTICALS CO., LTD. The sequence listing filed with the application follows.

SEQUENCE LISTING (32 sequences)

SEQ ID NO: 1 - protein, 25 aa, synthetic construct
  source 1..25: note = MY9286 FR1
EVQLLESGGGLVQPGGSLRLSCAAS

SEQ ID NO: 2 - protein, 10 aa, synthetic construct
  source 1..10: note = MY9286 CDR1
GFTFSDYTMT

SEQ ID NO: 3 - protein, 15 aa, synthetic construct
  source 1..15: note = MY9286 FR2
WVRQAPGKGLEWVST

SEQ ID NO: 4 - protein, 8 aa, synthetic construct
  source 1..8: note = MY9286 CDR2
VNPDGDST

SEQ ID NO: 5 - protein, 38 aa, synthetic construct
  source 1..38: note = MY9286 FR3
FYRDSVKGRFTISRDNAKNTLYLQLSSLKTEDTAMYYC

SEQ ID NO: 6 - protein, 12 aa, synthetic construct
  source 1..12: note = MY9286 CDR3
TKASLITWPQSP

SEQ ID NO: 7 - protein, 11 aa, synthetic construct
  source 1..11: note = MY9286 FR4
RGQGTLVTVSS

SEQ ID NO: 8 - protein, 119 aa, synthetic construct
  source 1..119: note = MY9286 VHH
EVQLLESGGGLVQPGGSLRLSCAASGFTFSDYTMTWVRQAPGKGLEWVSTVNPDGDSTFYRDSVKGRFTISRDNAKNTLYLQLSSLKTEDTAMYYCTKASLITWPQSPRGQGTLVTVSS

SEQ ID NO: 9 - DNA, 357 bp, synthetic construct
  source 1..357: mol_type = other DNA; note = MY9286 nucleotide sequence
gaggtgcagctgctggagagcggcggcggcctggtgcagcccggcggcagcctgaggctgagctgcgccgccagcggcttcaccttcagcgactacaccatgacctgggtgaggcaggcccccggcaagggcctggagtgggtgagcaccgtgaaccccgacggcgacagcaccttctacagggacagcgtgaagggcaggttcaccatcagcagggacaacgccaagaacaccctgtacctgcagctgagcagcctgaagaccgaggacaccgccatgtactactgcaccaaggccagcctgatcacctggccccagagccccaggggccagggcaccctggtgaccgtgagcagc

SEQ ID NO: 10 - protein, 25 aa, synthetic construct
  source 1..25: note = MY9293 FR1
EVQLLESGGGLVQPGESLRLSCEVS

SEQ ID NO: 11 - protein, 10 aa, synthetic construct
  source 1..10: note = MY9293 CDR1
GHTHTNYCMG

SEQ ID NO: 12 - protein, 15 aa, synthetic construct
  source 1..15: note = MY9293 FR2
WFRQAPGKGLEGVAA

SEQ ID NO: 13 - protein, 7 aa, synthetic construct
  source 1..7: note = MY9293 CDR2
IDTDGST

SEQ ID NO: 14 - protein, 38 aa, synthetic construct
  source 1..38: note = MY9293 FR3
TYADSVKGRFTISKDNAKNTLYLQMNSLKPEDTAMYYC

SEQ ID NO: 15 - protein, 29 aa, synthetic construct
  source 1..29: note = MY9293 CDR3
MAEDFRDEYAPEPRLSSGGYCSIGYGMDY

SEQ ID NO: 16 - protein, 11 aa, synthetic construct
  source 1..11: note = MY9293 FR4
WGKGTLVTVSS

SEQ ID NO: 17 - protein, 135 aa, synthetic construct
  source 1..135: note = MY9293 VHH
EVQLLESGGGLVQPGESLRLSCEVSGHTHTNYCMGWFRQAPGKGLEGVAAIDTDGSTTYADSVKGRFTISKDNAKNTLYLQMNSLKPEDTAMYYCMAEDFRDEYAPEPRLSSGGYCSIGYGMDYWGKGTLVTVSS

SEQ ID NO: 18 - DNA, 405 bp, synthetic construct
  source 1..405: mol_type = other DNA; note = MY9293 nucleotide sequence
gaggtgcagctgctggagagcggcggcggcctggtgcagcccggcgagagcctgaggctgagctgcgaggtgagcggccacacccacaccaactactgcatgggctggttcaggcaggcccccggcaagggcctggagggcgtggccgccatcgacaccgacggcagcaccacctacgccgacagcgtgaagggcaggttcaccatcagcaaggacaacgccaagaacaccctgtacctgcagatgaacagcctgaagcccgaggacaccgccatgtactactgcatggccgaggacttcagggacgagtacgcccccgagcccaggctgagcagcggcggctactgcagcatcggctacggcatggactactggggcaagggcaccctggtgaccgtgagcagc

SEQ ID NO: 19 - protein, 25 aa, synthetic construct
  source 1..25: note = HSA HuNb3-11 FR1
EVQLQESGGGLVEPGGSLRLSCVAS

SEQ ID NO: 20 - protein, 10 aa, synthetic construct
  source 1..10: note = HSA HuNb3-11 CDR1
GFTFQHYAMS

SEQ ID NO: 21 - protein, 15 aa, synthetic construct
  source 1..15: note = HSA HuNb3-11 FR2
WVRQAPGKGLEWVSS

SEQ ID NO: 22 - protein, 8 aa, synthetic construct
  source 1..8: note = HSA HuNb3-11 CDR2
ISMVGGGT

SEQ ID NO: 23 - protein, 38 aa, synthetic construct
  source 1..38: note = HSA HuNb3-11 FR3
SYADSVKGRFTMSRDNAKNTLYLQLNSLKSEDTAMYYC

SEQ ID NO: 24 - protein, 11 aa, synthetic construct
  source 1..11: note = HSA HuNb3-11 CDR3
VRGWHPDVPRP

SEQ ID NO: 25 - protein, 11 aa, synthetic construct
  source 1..11: note = HSA HuNb3-11 FR4
LGQGTLVTVSS

SEQ ID NO: 26 - protein, 118 aa, synthetic construct
  source 1..118: note = HSA HuNb3-11 VHH
EVQLQESGGGLVEPGGSLRLSCVASGFTFQHYAMSWVRQAPGKGLEWVSSISMVGGGTSYADSVKGRFTMSRDNAKNTLYLQLNSLKSEDTAMYYCVRGWHPDVPRPLGQGTLVTVSS

SEQ ID NO: 27 - DNA, 354 bp, synthetic construct
  source 1..354: mol_type = other DNA; note = HSA HuNb3-11 nucleotide sequence
gaagttcaattacaagagtccggtggtggtttggttgagccaggtggttctttgagattgtcctgtgttgcttctggtttcactttccaacattacgctatgtcttgggttagacaagctccaggaaagggtttggagtgggtttcttctatttctatggttggtggtggtacttcttacgctgactctgttaagggtagattcaccatgagtagagataacgctaagaacactttgtacttgcaattgaactctttgaaatctgaggacactgctatgtactactgtgttagaggttggcaccctgatgttccaagaccattgggtcaaggtactttggttactgtttcttct

SEQ ID NO: 28 - protein, 20 aa, synthetic construct
  source 1..20: note = GS20 linker
GGGGSGGGGSGGGGSGGGGS

SEQ ID NO: 29 - protein, 413 aa, synthetic construct
  source 1..413: note = MY9217 nanobody
EVQLLESGGGLVQPGGSLRLSCAASGFTFSDYTMTWVRQAPGKGLEWVSTVNPDGDSTFYRDSVKGRFTISRDNAKNTLYLQLSSLKTEDTAMYYCTKASLITWPQSPRGQGTLVTVSSGGGGSGGGGSGGGGSGGGGSEVQLQESGGGLVEPGGSLRLSCVASGFTFQHYAMSWVRQAPGKGLEWVSSISMVGGGTSYADSVKGRFTMSRDNAKNTLYLQLNSLKSEDTAMYYCVRGWHPDVPRPLGQGTLVTVSSGGGGSGGGGSGGGGSGGGGSEVQLLESGGGLVQPGESLRLSCEVSGHTHTNYCMGWFRQAPGKGLEGVAAIDTDGSTTYADSVKGRFTISKDNAKNTLYLQMNSLKPEDTAMYYCMAEDFRDEYAPEPRLSSGGYCSIGYGMDYWGKGTLVTVSSA

SEQ ID NO: 30 - DNA, 1239 bp, synthetic construct
  source 1..1239: mol_type = other DNA; note = MY9217 nucleotide sequence
gaagttcaattgttggaatctggtggtggtttggttcaaccaggtggttctttgagattgtcttgtgctgcttctggtttcactttctctgattacactatgacttgggttagacaagctccaggtaaaggtttggaatgggtttctactgttaacccagatggtgactctaccttctacagagattctgttaagggtagattcaccatttctcgtgataacgctaagaacactttgtacttgcaattgtcctctttgaaaactgaagatactgctatgtactactgtactaaggcttctttgattacttggccacaatctccaagaggtcaaggtactttggttactgtttcttctggtggaggaggttccggtggaggtggttctggaggtggtggttctggtggtggaggttctgaagttcaattacaagagtccggtggtggtttggttgagccaggtggttctttgagattgtcctgtgttgcttctggtttcactttccaacattacgctatgtcttgggttagacaagctccaggaaagggtttggagtgggtttcttctatttctatggttggtggtggtacttcttacgctgactctgttaagggtagattcaccatgagtagagataacgctaagaacactttgtacttgcaattgaactctttgaaatctgaggacactgctatgtactactgtgttagaggttggcaccctgatgttccaagaccattgggtcaaggtactttggttactgtttcttctggaggtggaggatcaggaggaggtggttctggaggaggtggatctggtggtggaggatctgaggttcaattgttggaatctggtggtggtttggttcaaccaggtgagtctttgagattgtcttgtgaggtttctggtcacactcacactaattactgtatgggttggttcagacaagctccaggaaagggtttggaaggtgttgctgctattgatactgacggttctactacttacgctgattctgttaagggtagattcactatttctaaggataacgctaagaacactttgtacttgcaaatgaactctttgaagccagaggatactgctatgtactactgtatggctgaagatttcagagatgaatacgctccagagccaagactttcttctggtggttactgttctattggttacggtatggattactggggtaaaggtactttggttactgtttcttctgct

SEQ ID NO: 31 - protein, 413 aa, synthetic construct
  source 1..413: note = MY9219 nanobody
EVQLQESGGGLVEPGGSLRLSCVASGFTFQHYAMSWVRQAPGKGLEWVSSISMVGGGTSYADSVKGRFTMSRDNAKNTLYLQLNSLKSEDTAMYYCVRGWHPDVPRPLGQGTLVTVSSGGGGSGGGGSGGGGSGGGGSEVQLLESGGGLVQPGGSLRLSCAASGFTFSDYTMTWVRQAPGKGLEWVSTVNPDGDSTFYRDSVKGRFTISRDNAKNTLYLQLSSLKTEDTAMYYCTKASLITWPQSPRGQGTLVTVSSGGGGSGGGGSGGGGSGGGGSEVQLLESGGGLVQPGESLRLSCEVSGHTHTNYCMGWFRQAPGKGLEGVAAIDTDGSTTYADSVKGRFTISKDNAKNTLYLQMNSLKPEDTAMYYCMAEDFRDEYAPEPRLSSGGYCSIGYGMDYWGKGTLVTVSSA

SEQ ID NO: 32 - DNA, 1239 bp, synthetic construct
  source 1..1239: mol_type = other DNA; note = MY9219 nucleotide sequence
gaagttcaattacaagagtccggtggtggtttggttgagccaggtggttctttgagattgtcctgtgttgcttctggtttcactttccaacattacgctatgtcttgggttagacaagctccaggaaagggtttggagtgggtttcttctatttctatggttggtggtggtacttcttacgctgactctgttaagggtagattcaccatgagtagagataacgctaagaacactttgtacttgcaattgaactctttgaaatctgaggacactgctatgtactactgtgttagaggttggcaccctgatgttccaagaccattgggtcaaggtactttggttactgtttcttctggaggtggaggatcaggaggaggtggttctggaggaggtggatctggtggtggaggatctgaagttcaattgttggaatctggtggtggtttggttcaaccaggtggttctttgagattgtcttgtgctgcttctggtttcactttctctgattacactatgacttgggttagacaagctccaggtaaaggtttggaatgggtttctactgttaacccagatggtgactctaccttctacagagattctgttaagggtagattcaccatttctcgtgataacgctaagaacactttgtacttgcaattgtcctctttgaaaactgaagatactgctatgtactactgtactaaggcttctttgattacttggccacaatctccaagaggtcaaggtactttggttactgtttcttctggaggtggaggatcaggaggaggtggttctggaggaggtggatctggtggtggaggatctgaggttcaattgttggaatctggtggtggtttggttcaaccaggtgagtctttgagattgtcttgtgaggtttctggtcacactcacactaattactgtatgggttggttcagacaagctccaggaaagggtttggaaggtgttgctgctattgatactgacggttctactacttacgctgattctgttaagggtagattcactatttctaaggataacgctaagaacactttgtacttgcaaatgaactctttgaagccagaggatactgctatgtactactgtatggctgaagatttcagagatgaatacgctccagagccaagactttcttctggtggttactgttctattggttacggtatggattactggggtaaaggtactttggttactgtttcttctgct